European Patent Specification EP 3 662 069 B1, published August 30, 2023. Title: New bio-pesticides for controlling plant pests. Applicant: Univerza v Ljubljani Kmetijski institut Slovenije. The sequence listing filed with the application follows.

SEQUENCE LISTING (5 sequences)

SEQ ID NO: 1 - protein, 138 aa, Pleurotus ostreatus
MAYAQWVIIIIHNVGSQDVKIKNLKASWGKLHADGDKDAEVSASNYEGKIVKPDEKLQINACGRSDAAEGTTGTFDLVDPADGDKQVRHFYWDCPWGSKTNTWTVSGSNTKWMIEYSGQNLDSGALGTITVDTLKKGN

SEQ ID NO: 2 - protein, 138 aa, Pleurotus eryngii
MAYAQWVIIIIHNVGSKDVKIVNLKPSWGKLHADGDKDTEVSASKYEGTVIKPDEKLQINACGRSDAAEGTTGTFDLVDPADGDKQVRHFYWDCPWGSKANTWTVSGSNTKWMIEYSGQNLDSGALGTITVDTLKKGN

SEQ ID NO: 3 - protein, 138 aa, Pleurotus eryngii
MAYAQWVIILIHNVGQQNVKIKNLNASWGKLYADGDKDTEVPASKYEGMVIAPDDQVQINACGREDAAEGTTGTFDLVDPNDSDKQVRHFAWDCPWGTKANSWVVGGSNSKWMIEYTGQNLDSGALGTITVNTLRIGN

SEQ ID NO: 4 - protein, 523 aa, Pleurotus ostreatus
MEAVLSRQAATAEAIGRFQDSSTSVGLVAGSPSTRIRRQADNVVLKSTSQAGDTLNDVIQDPTRRNKLINDNNLLKGIIMGRDGPVPSSRELIVRPDTLRAIINNRATIETTTMEAEFTETLMESNYNSASVKVSAPFITANSEYSESSSFKNTETEKSMYTSSRYLFPQGRIDFTTPDSGFDDVIKLSPQFTSGVQAALAKATGTEKREALQNLFQEYGHVFRTKVHIGGVLSAHTMETFSRSENETEVKQDVKAGLEGAVKGWGGGATAGHGNTQGTITTSQNRKLNVKYIVNGGDYTKIQNTEEWVASTNQSEHWRVIEVTEVTAVADLLPQPIRGQVKDLLKPLLGKWVDVEKVPGLESLPVSVYRPKGAIPAGWFWLGDTADASKALLVKPTLPARSGRNPALTSLHQGSGMTEQPFVDLPQYQYLSTYFGSFAHDTPPGSTLRGLRPDHVLPGRYEMHGDTISTAVYVTRPVDVPFPEDECFDLKSLVRVKLPGSGNPPKPRSALKKSMVLFDSGEK

SEQ ID NO: 5 - protein, 522 aa, Pleurotus eryngii
MAAVLSRQAATAEAVERFQDSSTSVGLVAGSPSRIRRQADNVVLKSISQAGDTLNDVIQDPTRRNKLINDNNLLKGIIMGRDGPVPSSRELIERPDTLRAIINNRATIETTTVEAEFTETLMESNYNSASVKVSAPFVTANSEYSESSSFKNTETEKSMYTSSRYLFPQGRIDFTMPDSGFDDVIKLSPQFTSGVQAALAKATGTEKREALQDLFLEYGHVFRTKVHIGGVLSAHTMETFSRSENETEVKQDIKAGLEGAVKGWGGGATAGHGNTQGTITTSQNRKLDVKYIVNGGDYTKIQNTEEWVASTNQSEHWRVIEVTEVTAVADLLPQPIRGQVKDLLKPLLGKWVDVEKVPGLESFPVSVYRPKDAIPAGWFWLGDTADASKALLVKPTLPARSGRNPALTSLHESSGMTEQPFVDLPQYQYLSTYFGSFAYDTPPGSTLRGLRPDHILPGRYEMHGDTIGTAVYVTRPVDVPFPEDECFDLKSVVRVKLPGSGNPPKPRWALKKSMVLFDSGEE